European Patent Specification EP 3 581 660 B1, published June 7, 2023. Title: NICHE TARGETING OF QUIESCENT CANCER STEM CELLS. Applicant: The Regents of The University of California Jamieson, Catriona Goeff, Donald Smitg, Kristen. Application EP 12847894.8. The sequence listing filed with the application follows.

SEQUENCE LISTING (14 sequences)

SEQ ID NO: 1 - DNA, 20 bp, artificial
  BCL 2L Forward  Primer
atgtgtgtggagagcgtcaa

SEQ ID NO: 2 - DNA, 21 bp, artificial
  BCL 2L Reverse Primer
ttcagagacagccaggagaaa

SEQ ID NO: 3 - DNA, 19 bp, artificial
  MCL L1 Forward Primer
agaccttacgacgggttgg

SEQ ID NO: 4 - DNA, 20 bp, artificial
  MCL L1 Reverse Primer
aatcctgccccagtttgtta

SEQ ID NO: 5 - DNA, 20 bp, artificial
  MCL 1S Forward Primer
gaggaggacgagttgtaccg

SEQ ID NO: 6 - DNA, 20 bp, artificial
  Reverse Primer MCL 1S
actccacaaacccatccttg

SEQ ID NO: 7 - DNA, 20 bp, artificial
  Forward Primer BCL XL
catggcagcagtaaagcaag

SEQ ID NO: 8 - DNA, 20 bp, artificial
  Reverse Primer BCL XL
gaaggagaaaaaggccacaa

SEQ ID NO: 9 - DNA, 18 bp, artificial
  Forward Primer BFL 1L
gctgggaaaatggctttg

SEQ ID NO: 10 - DNA, 21 bp, artificial
  BFL 1L Reverse Primer
tcagaaaaattaggccggttt

SEQ ID NO: 11 - DNA, 20 bp, artificial
  BCR ABL Forward Primer
ctccagactgtccacagcat

SEQ ID NO: 12 - DNA, 20 bp, artificial
  BCR ABL Reverse Primer
ccctgaggctcaaagtcaga

SEQ ID NO: 13 - DNA, 21 bp, artificial
  HPRT Forward Primer
cgtcttgctcgagatgtgatg

SEQ ID NO: 14 - DNA, 21 bp, artificial
  HPRT Reverse Primer
tttatagccccccttgagcac